European Patent Application EP 4 293 113 A2, published December 20, 2023. Title: EXPRESSION INHIBITOR OF INFLAMMATION PROMOTING FACTOR, SCREENING METHOD FOR ACTIVE INGREDIENT THEREOF, EXPRESSION CASSETTE USEFUL FOR SAID METHOD, DIAGNOSTIC AGENT AND DIAGNOSIS METHOD. Applicant: National University Corporation Tokyo Medical and Dental University. Application EP. The sequence listing filed with the application follows.

SEQUENCE LISTING (48 sequences)

SEQ ID NO: 1 - DNA, 446 bp, Homo sapiens
  source 1..446: mol_type = other DNA
catgggcacctcagattgttgttgttaatgggcattccttcttctggtcagaaacctgtccactgggcacagaacttatgttgttctctatggagaactaaaagtatgagcgttaggacactattttaattatttttaatttattaatatttaaatatgtgaagctgagttaatttatgtaagtcatatttatatttttaagaagtaccacttgaaacattttatgtattagttttgaaataataatggaaagtggctatgcagtttgaatatcctttgtttcagagccagatcatttcttggaaagtgtaggcttacctcaaataaatggctaacttatacatatttttaaagaaatatttatattgtatttatataatgtataaatggtttttataccaataaatggcattttaaaaaattcagcaaaaaaaaaaaaaaaaaaa

SEQ ID NO: 2 - protein, 407 aa, Homo sapiens
MLLSVTSRPGISTFGYNRNNKKPYVSLAQQMAPPSPSNSTPNSSSGSNGNDQLSKTNLYIRGLQPGTTDQDLVKLCQPYGKIVSTKAILDKTTNKCKGYGFVDFDSPSAAQKAVTALKASGVQAQMAKQQEQDPTNLYISNLPLSMDEQELEGMLKPFGQVISTRILRDTSGTSRGVGFARMESTEKCEAIITHFNGKYIKTPPGVPAPSDPLLCKFADGGPKKRQNQGKFVQNGRAWPRNADMGVMALTYDPTTALQNGFYPAPYNITPNRMLAQSALSPYLSSPVSSYQRVTQTSPLQVPNPSWMHHHSYLMQPSGSVLTPGMDHPISLQPASMMGPLTQQLGHLSLSSTGTYMPTAAAMQGAYISQYTPVPSSSVSVEESSGQQNQVAVDAPSEHGVYSFQFNK

SEQ ID NO: 3 - DNA, 8504 bp, Homo sapiens
  source 1..8504: mol_type = other DNA
gagctcattctctgcccgcagccccccttcatctctctcctcctgctccttttctcctcctttctcctccccctcccttttttcctccctccctctccccctttccctcgctcccctcctccctccctccccgtctttcttaccccctccctttctctctctctctctctctcgctcgttccctaacattaaagagaaaatgctgctatccgtgacttccaggcccgggatttcgacttttggctacaatagaaacaacaagaagccatatgtgtcattggctcagcagatggcaccacctagcccaagcaacagtacacctaacagcagtagtggaagcaatggaaatgaccagctgagcaaaaccaacctatacatccgaggattgcaaccaggcactactgaccaagatcttgtcaagctgtgtcagccatatggcaagattgtttccactaaggccatactggacaagaccacaaacaaatgtaaaggctatggctttgtagattttgacagcccttcagcagcacagaaagctgtaacagcactgaaggccagcggtgtacaggcacagatggcaaagcaacaggaacaggaccccacaaatttatacatctcaaacctcccactgtcaatggatgagcaggaactggaggggatgctgaagccctttggccaggttatctccacccgtatccttcgagataccagtgggaccagcagaggtgttggctttgcaaggatggagtccacagagaagtgtgaagccatcatcacccactttaatggaaaatatattaagacaccccctggagtaccagccccatccgatcccttgctttgcaaatttgctgatggcgggccaaagaaacgacagaaccaaggaaaatttgtgcaaaatggacgggcttggccaaggaatgcagacatgggcgtcatggccttgacctatgaccccaccacagctcttcagaatgggttttacccagccccctataacatcacccccaacaggatgcttgctcagtctgcactctccccatacctttcctctcctgtgtcttcgtatcagagagtgactcagacatctcctctacaagtacctaacccatcctggatgcaccaccattcatacctcatgcagccttcaggttcagttctgacaccagggatggaccatcccatttctctccagcctgcctccatgatgggaccccttacccagcaactgggccatctctccctcagcagcacaggcacgtatatgccgacggctgcagctatgcaaggagcttacatctcccagtacacccctgtgccttcttccagtgtttcagtcgaggagagcagcggccaacagaaccaagtggcagtggacgcaccctcagagcatggggtctattctttccagttcaacaagtaacagtgggattcccctccccatctttactgaatagaaatgaattcttggagatactcatgctcccagattccagagggttaaccaggaatggagaccatccgtcggccctgctaaggactaacacttagccatcgtttttcacaggcctgggcctggaaaaagaaatctctacgttcctgccctttactattgctgatggagcctgggggaaccatcactttttttgtgtgctacattcaaggagatcaaaaaaacttttcttcttttgcaaagaaagctttttgtttttaactgcaacgtacttttcccctaccttgaagagacatggtggtcgcagcttctcatctatatgaaaaagttttcgatgtattggaattatttgggaatgcttttaaaacaatttgtaattatttctttacaaaccaaaacagaacagaaaggtgtggtgctggaacatcgatgaaggagccctacttactgagcttagttatggacttttttgatgcatgtgtgtatgtgttttaaaaagtatgcaggctctaaaaatgttattttgtaaagctctcagctcatgcaccccatctcctcttcacccatattatgccttctttctcttgtccagattcttctttttctcttttctaaacagctgagcctgcctactttgcccttttacagcttttaattttatggatttttaaaaatgaaatttcatgtggaatttggggttggggggcaggctgggcaaggaacaaggcagaacactaagtaggccatggaagtggctgttctttcccccaccctgccacaccctgggagaaaaaactagactttggcttcagaaagcacagatgtgacccaggcttactaaagagacaactccacagccctgggaacacacccttgagccaaacttggttgaagactaggtcttccctggcaagttccggaagaatggacttactgacttttatcaactcttctcactgccaaggccaacagcatctgaggtatagctttttgggagtacctgctttcttgcctcctggaggatattttctgtcctgggcttcatggcccctctcttccctgttacacattgctgtgctcagagcctttgcagctgcgacctagttgaatccacataggctccttccacacggtggaagatctgctgcttcactcacagaccaggagttctcaatcagaggtggttttgtccctcaggcctttggcaacatctagagacagttttgattgccacgcctggaggtgggatgtgtgtgctactggcatctagtggctgctaaacatcctacactgcataggatagtccccactacccccagccaagaattatctgactccaggggtcaatattgccaagactgggaaacactgatatagacagtgttgtccctgcctcctgggttagggtaaattttcaccccaaccctggacaaacagtgccttttgacactcatgcaactgttggggaaggactggactgggatccttgaattctccccagactttgacttttgataactctgcatatagcaagagtgattcttgaaagagctgtggctccatgctgaatgcacacatgtactcagagggattcaggtgggcattgttctggtgtgtgctgtgcaatggtgggaaaggacaaagctctctaaactgtccagagcaacctgccctgccccggtgtgcttggaccctttgcccagggaaccaggacatcagaaataatgttccttctgtggaaggacaacggggagctagggtagcaaagagcaataaattccaactctttatgaggtcaggagtcctttaaaaaagcctatgtcttggtctttaactgtccccttctgcaagatgtgactctatacacatggagacagattgaagaaagacttcacccatcttctaggaaataaaatcctgctcttgtcttctcccagtcactcccttatgcactgaaaggagaatttgactcccttgcacttcaaggccaggtgcctctccactagacagtcagacaaaggcaaataatggaggatagagagacaggtgttcattaggctggccatagggagaggaagggggtgacagcaggggaaaagaaactgtagtatcagttgtcacaagtagagctcggcccagctttccctcccttcccagccaccctagaattgagagtcccagtgcccctagtgtcgactttctatgtacatcctaggggtgagggagtgcggggcaatgggtaggatataaagcgtaaaggacaaattgccgcagtcttctaattgatgcttccaaactcaggaagggcttatccagtgtaaaatagccccaagcccagcaaccttctagagggctctggctgggcagatagcttttgtttttgagtctccagccctcagtcaaggaaaatataccatagctgctttcttgtcagtggcctttgagagaaagagaaaacaaatctagaattctgttcatctgatagaccgggggagctttgctatggtaggaggtttaggaagggcctttcacgcatagaaaccattgttgatattgccactcccctctcctctgcctcacagaactcctgattctgtcttctttctctctctatatatatattttaaaatgtttaaatggctctaattttttgttttgaattttgaatttaccttttggagttcttctcatgtgaatctacttgttagattgtattaatgagtgtttctggtttgggcatgggaagtgatgggggcctgaagttattttgcagtggctaatggcactgaggaatttcttttttggtgcatttggtttacactcatttcctctcctaattgttagttcatttgtaacagtgggtgagtgtttggaggaaaggagggagaagaaaggagggatactgtttctcccatgaaatagtctaattggttgggttgatggcagaaggaaacataggggagccttccagctcacagccaagggttgggctcttaaacactatgcctagtgttttctgaatgctgtcttcatggagcccagctcttactctctttgtactttacatctcacccccactcattacagatgctcataacattcttaaaatattttagtacttggcatttttctgttttcagtcagctagaacacactagagtcctttcctcagatggcataatcctttataggctctgagcctgcctagccatctcctatcggtgttattactcctcatctcaggctctgagatgatactcagaccctaaactgattggactttttggaggagggtgccagtagagaggtcaggaagatgtggagatgatgatggagagagatgtttttattttattttattttttcagacagagtcttgctctgtcgcccaggctggagtgcaatggcacgatctcggctcactgcaacctccgcctcccaggttcaagcaattctcctgcctcagcctcccatgtagctgggattacaggcacccaccaccatgcccggctaatttttttatttttagtagagatggggtttcaccatgttggccaggctggtctcgaactcctgacctcaggtgatctgcccgccttagcctcccaaagtgctgggattacaggcgtgagccaccgcgcccggcctttattttattttttagagatggtcttgctgtgtcacccaggctggagtgcagtgatgcagtcgtagtctactacagtcttgaattcctgggcccaagggttcttcccacctaagcctcccaagtagctggaagtacaggcacatactaccaagcccagttcgttattttaagtttttgtagagacaggggtcttactatgttgcccagactggtcttgaactcctgtcaagtgagcctcccacctcagcctcccaaagtgctatgattacaggtgtgagcctccatgcttggatgagatgttgtttttaatgtttttggttttttggttttgttgttttgtttttttgagacagggtctcactctgtggcccaggctggagtgcagtggcaccataatggctcactgcagcctcgacctcccaaggctcaggtgatcctcttgcctcagccaccccttccccggccaccaagtagctgggactatgggcttgtgccaccatgcctggctaatttttttatttttagtagagatggggttttaccacgttggccaggctagtgtccaactcctgacctccaaacagctaatttttgtatttttaatagagacaggttttcgccatgttgcccagcctcgtctcgaactcctgggctcaaatgatccacccacctcggcctcccaaagtgctgggattataggcatgagccaccacacctggccttttcagtttttttatttttattttttctttgagacggagtctcgctctgtcgcccaggctggagtgcagtggcgtgatcttggctcactgaaacctccatctcctgggttcaagcagttctcctgcctcagcctcctgagtagctgggattacaggtgcctgccaccatgcctggctaatttttgtatttttagtagagacagggttttgccacattgcccaggctggtgttgaactcctgggctcaaatgatccacctgccttggcctcccaaagtgctgggattacaggcgtgagccactgcacccggccctttgtagtgtttttaactaaagaatttgtagagttgcccaggccaggaagcctggtggctctaaagggtaatagaccttgtcagtaacagataaggagtggtaagaggacattactcatattgaagatgaagaccagactttgctgcttcacaggccatgcgctgggttgggccacttcagctccactccattcgttttcctttcctaacttgacaatcagctcactcaccctcccttagtgcctccagtgcctactcctgtcactccaatgtcaacccattgggagttgaggcctgtcactccaatgtcaacccgtgggctgttactttgcgtcatatgatgctgtgagaggccttgctggaatgtcctaggaatccctagtagcagtggctattagtcttctagaaaagaactattgctgctgccttgtgcacatgccccaccttctgggcaagtggcagcattgcgctcatgaggggctttgcattcttagccaagggcaataaactgggtgggtgatctggcccaaacttgcccctaggctctgctagccctgaatcagcaggcttcagagacgagggtgggtgttataaaagccagtctgtaaagggtaaattccaaatcttgtgccttgttataccaatccttcctgattcccgtttaaaccaactactctatttctgtgctgcctacattttcaatcctcccacgcattagcaaattcctgaaatttcctcatttggtaggccttccataggagtcagctatggacttccataggagttggcagctaaaaccagactgtgagcttctgtctccgttctgatttttgctgcacctcccaggggacagtccccacatgattacaaaagccaggtgccctcatcacccgttacccctgacctgtccacttgttttgaataaaccttcattctccaagcagatccccaaacttccttgtccttgttacacgtctacctcacaacctcacaattcaacaacaggtaaatacctggattcactgatttctttactgtccttctctgagggttgggaaggtgggggctagaaaaggctcataatttttaaactcttgggaattaaacttgggaatttctattcctacagtgttttctctgggatttttagctcactgatcgccctagaatagtgtgaactctccagataggtcctgctgtgataggccaggggagtaggctgtgcagtgacggcttagggtaataagtaatggttggaggacaccagcataggagcagagtttagaacttaagaggacaagaaagctgctcagtggctggcgtatagctgtgaaggtaaccaaacaccaaagagggagtctgtcatttttataaggctggaagcgaatgttccttttctaccttaacatacagtttagggggttgcaccaagacaaagtttccaggctggagggtaatacatatccagcgcgagtgaagtccccactccaacatataccctttttgggtgggtaaacacctctttgcatgtggacagaaaatgtttatacttaaacagacatattttgcatatttttatctggagacttcttctagttttatactcttcccacatctatgccaatgccaccattctaaaacttacactccttttctacccctggtcttttccttgtccttccctacaacttggtagaggtccattttgtcttacttcacacttttttttttttaaataaaacacaaaagtctacgtcttggtgtcttatccgtgagtgggaagtggtaagctggtgatggtcccatatttgctatgacaggaacacagaggtggcagcttaggaagctggggccacatctcacaaggcaggacctggatgcactgaatccccctttgctccagcaactcagccagacatttaggcaggagcactaatgaccctttccatccacacagagggtatggaacaggagcccctgttgttcccttgcctgtggtctcttaagccagtcatacctatcccaacgccgtctccccctcaggtgtgtagaagggaagatgaatacacagagtcttttgaatctctatcaaatgtggttttttttattcaacaactgacaagcacttttctacagctgcacttgtggaacatcacatggcaaaaacaggagttttttcgctagactttttttttctttttaaccttattaaaaatgagattggtcctaaaaatatagaaagaaataaatttaaattcacaaaaaactgtacattatcaaaaagtcactaaaacaccacatttggttatataaaaagtcccttttgctgtaaaaggaacacagaaacttaaaaaaaaaaaaaaaaaa

SEQ ID NO: 4 - DNA, 5207 bp, Mus musculus
  source 1..5207: mol_type = other DNA
ctttctcctccccctcccttctcccttccctccctctttccctcccttcctctctccctctcctttccccctcccctcctccctccctctttctccctccctttccttcactctcttctttctctctctcagctccgtaacagtaaagaaaaaatgctgctatcagtgacttccaggcctgggatttcgacttttggctataacaagaacaacaagaagctatatgtggctcagcaaatggcacctccaagtccaaggaatagcacccccaacagcagcggcggaggcggcggcgggagtggtgggaacgaccagctgagcaaaaccaacctgtatatccgaggactgcagccaggcaccactgaccaggaccttgtcaagctctgtcagccgtatggcaagattgtctccactaaggccatcctggacaagaccacaaacaagtgcaaaggctatggctttgtggacttcgacagtccgtcatcagcacagaaagctgtaactgcactgaaagccagtggtgtgcaggcacaaatggcaaagcaacaggagcaagaccctacaaacttatacatctcaaacctccctctgtcaatggacgagcaggaactggaggggatgctgaagccctttggccaggtcatctctactcggatccttcgagacactagtggggccagcagaggggtcggctttgcaaggatggagtcaacagagaagtgtgaagccatcatcacccactttaatggaaagtatataaagacaccccctggagtagcagcaccttctgaccctttgctttgcaaatttgctgacggtgggccaaagaaacgacagagccaaggaagatacgtgcaaaatggacgggcctggccaaggaacggagacatgggcggtatggccttgacctatgaccccactgctgcccttcagaatgggttctacgcagctccttacagtatcgcccacagcaggatgcttgctcaatctgcgctagccccgtatcttccatctcctgtgtcttcctatcagggctcagttctgacaccagggatggaccaccccctctctctccagcctgcctccatgatgggacctcttacccagcaactgggtcacctgtcactcaacagtctgggcacgttcatgccggcagctgctgctatgcatggggcttacatctcccagtacccagctgtgccttcttccagtgtttctgctgaggagagcaatggccagcagaatcaactggcagtggagcccccctcagaccacggggtctatcctttccagttcagcaaataatgaggtccagacctggggagagaagcctatgcagtcctccttgggctccttcctgtggctgatggaacctgaggaatcacgttggtttttttttttgaatgtgctacattcaagatcaaaaagacttttttttcttttgcaaaagaagtttcttgctttgtatttaattgcagcgaacctttctcctaccccaaagacaccagttgaggtgcttctcatcttcgagaggtttgggtatgttgggcttttaaaatggtttaagaacaatcgcagtgctgtgaagtcagtgaaggggcgctgcttgccaggttcagttagggactattttcaatgtgtgttttagatatgcaggcttaaaacttttgttttgcaaagctctcaacacacactttgcacacacccacccacctccctcccacgcactgtttaaggcagggtctcacagtgcagtcctggctggctgacaatgtagaccaggctggctttgaactcagcgatccttcccactctgtctgagtgcaccgccatgcctagctagttgtttttttttttttggttttttttttttcaagacagggtttctctgtgtagccctggctgtcctggcgctcactttgtagaccaagctagcctcgaacttagaaatccacctgcctctgcctcccaagtgctgggattaaaggcgtgcgccaccaccgcccggctagttgttttttaaaacttctccacaatggtctttttttcttttccatttagcttagcctgcctactttgcctttttacaatttttaattttatgaatttgatttaaatttcatgtggaattgggggaagggagagcaacgcacaggtagagaagtgtggcagtagaggttgctttccctctgccctcctggcctaggaggggttagactttgacttcaggaagcagacatgtgacaaccatgcagcctttggaaaccaccttcaaccaactctggtggcaagtgccactgagaagtggcatccagcttcagcatcctggatacctgctctgcctcctggagggtcttgggtcttcatcctgccccaggtctcacagcccctgcccctgctgagcaagttctgccttccactttaccaggaggttgttttgtccccgagaggctgctgtcttgtccatcatcatccttgattaccaagcctggggagtatcatgtgtgctggtcctgaacacctgacagaacctggccccactcctccaccccttattccctggcagttatttggtgtagactaaaccccagtccagccttggacatggagcctgttagttcatgtacttggccagcagtgacatctgtgactttgcctcctggaggatcttttctgcctgggttctcacagcctctcatcccagctgcacatggctgtactcaagtggtacttggctgaatcacttaattcagcaggagccatcttatttagcagggctcacccttggttgtatgtacatgccaagtgcacacagtttgaagggatgaaagcaagaactgttgtgtatactgtgcatgcttgagaatggactgagctttctctatgcagcatacccagcccagccctggtgtttggaccccttccccagggaaccagaccaccagaaataattttccttcttgtggaaggacgacggggtgctaggatagaaaaaggcaagactcacagctccctggccactcaaaggtcaggagggacttgtaaacatgcctgccgttaactattcccttctgcaagactttcagcacaaaatgtgacttgttacatcacatcccttcacgtcataagtacacctccagtagacaaagcaatggagatggggaagtgtgtccagaggtcagtgtgaaagaggaagggcagggcatggtgatggtgagaaactggctcagcagctgtgcacactacagaattgggaatcctggcctgactgtgctgctgtgcgttctagactgaggaaggggctgaggacaatggacagcataaagtacaaaatgaccagttttctcattggtgcttccaacatcaggaaggtcatacccagttatcgacctctagccctctagcactcagtgacagactcagagctctgtcctgtggaaaccctgctgacagtcttgctgccactgctgctccttcactgcctattaaaaattgttcctttttctgtagttctaaagcaatttgaataactgacagttttaaaatttgaaattacctttttaggtttttcttttgagtatactggttagggttctagtgtttctggttgaacaggtgtgagcatgggaaatgagggcaacctgtaattttgtttttatagtggttaatggcactcactgtgtaatttctgcttagtgatttccatccactcttttcctcattagctcattactcagaaaggtagcgactgaagacaggaagtagtatgcaagccatgagggatgagttgtaagcctcctctccatcatcctgcccaaggctcctaacagtctcctgagtcctgtttgcatggaggccagatagatggctctgcactctatatctcacctgtactcattttagtacattgtggttttgcttccaatcaatcagagtggactagagctcacacctgacctcgtgtgactcttcactaggctccaggcctatcccatctcattgggtcagactgtagatggactggacttttggagacaggtcctgctattacttaggaatatgtgggaacaatgatagggaccaagcttgtgaagcaaaacggctttggaaagggcaagtgctcaataataaaaaatggggtggaagtgaagcgttatttgctgagggtttcggaaggactagtttgtttttgtccctggcccttccggtcaagtgggcacctcccattttgtcgccaagagcaatacagttgagtaggtggtagacccaaactcacccagccatttctagacctgaattcagaggataaggtgagtctagaggtatatacaaccaatgcttgttagaccaattcttaccaattcggagcaagccggtggctctacttctgggtaacctgcctcttaaaagtgcctttgatcccagtagtagattcagggtctacaggagccttccctcagcagctaaaaccaatttgtctcctctactctttgctgcacctcccggaggtggtctccatgtggcagtgatgccctcatcacccttgtgaccaccgctctgaatgttcaaaataagcatttcctgtccaagcaaatccctaaactccctcgtcctcattactcaactacctcagtctgacaactcaaggcacacaagcacctacttgcctcccaccatcctttactgcccttgtctttgtggggttggaacaaatgcaaactcctcagttccacaacccaaaactgctctttctggatcgtcttctccagtgacgttggctccctacaagagcgaactctccatatgggtcagtccctgtaggacaagccagggactatgctgtgcagtcaaatgccaggtttggagcatagcttaagaccgcagagagtaaggacttgagtggtggtggtgtgcagtttgagagagctggaatggacgtctctgctcctgccctctgggcgggtcgggtgatgacttctagatgcactccttaccctggagggaagttaatttatacttaagatgcattttgtacatttcccctttacccagaaacctgtagtttcatactcccatgtctatgccaacactacctatcgctcactctccgtggctgacttctggttccatttccttcctgtgacttggaagagctttacttttgctcacgtgaacctttcttttttaaataaaacacaaaagcctcc

SEQ ID NO: 5 - protein, 383 aa, Mus musculus
MLLSVTSRPGISTFGYNKNNKKLYVAQQMAPPSPRNSTPNSSGGGGGGSGGNDQLSKTNLYIRGLQPGTTDQDLVKLCQPYGKIVSTKAILDKTTNKCKGYGFVDFDSPSSAQKAVTALKASGVQAQMAKQQEQDPTNLYISNLPLSMDEQELEGMLKPFGQVISTRILRDTSGASRGVGFARMESTEKCEAIITHFNGKYIKTPPGVAAPSDPLLCKFADGGPKKRQSQGRYVQNGRAWPRNGDMGGMALTYDPTAALQNGFYAAPYSIAHSRMLAQSALAPYLPSPVSSYQGSVLTPGMDHPLSLQPASMMGPLTQQLGHLSLNSLGTFMPAAAAMHGAYISQYPAVPSSSVSAEESNGQQNQLAVEPPSDHGVYPFQFSK

SEQ ID NO: 6 - protein, 355 aa, Mus musculus
MAPPSPRNSTPNSSGGGGGGSGGNDQLSKTNLYIRGLQPGTTDQDLVKLCQPYGKIVSTKAILDKTTNKCKGYGFVDFDSPSSAQKAVTALKASGVQAQMAKQQEQDPTNLYISNLPLSMDEQELEGMLKPFGQVISTRILRDTSGASRGVGFARMESTEKCEAIITHFNGKYIKTPPGVAAPSDPLLCKFADGGPKKRQSQGRYVQNGRAWPRNGDMGGMALTYDPTAALQNGFYAAPYSIAHSRMLAQSALAPYLPSPVSSYQGSVLTPGMDHPLSLQPASMMGPLTQQLGHLSLNSLGTFMPAAAAMHGAYISQYPAVPSSSVSAEESNGQQNQLAVEPPSDHGVYPFQFSK

SEQ ID NO: 7 - DNA, 5390 bp, Mus musculus
  source 1..5390: mol_type = other DNA
acttcctgtcctgttggaaatgaaagttaggaattgggggtggtagccgtgcacgtatttattctgcagcatgccggcactgtctgtttcgttatcacagcaaagcagccgcaggaaaaacagagagcagagctttgttttagagagagtctgggcttgaggtctgttgtgacaaagacggagttaatttacttctggagaatgtgtgtggcagcagtgggaggcctgaggaggggctctgaaggcattcagtctccctccctgttctaggtggatggataggcttctttggtatcacttgtaagttttcttttcctgttccaactcctccttggagggcatattggagctcagagaggactctgtgaacgtcatttggcttggccataaattccacacctgctatatgtggctcagcaaatggcacctccaagtccaaggaatagcacccccaacagcagcggcggaggcggcggcgggagtggtgggaacgaccagctgagcaaaaccaacctgtatatccgaggactgcagccaggcaccactgaccaggaccttgtcaagctctgtcagccgtatggcaagattgtctccactaaggccatcctggacaagaccacaaacaagtgcaaaggctatggctttgtggacttcgacagtccgtcatcagcacagaaagctgtaactgcactgaaagccagtggtgtgcaggcacaaatggcaaagcaacaggagcaagaccctacaaacttatacatctcaaacctccctctgtcaatggacgagcaggaactggaggggatgctgaagccctttggccaggtcatctctactcggatccttcgagacactagtggggccagcagaggggtcggctttgcaaggatggagtcaacagagaagtgtgaagccatcatcacccactttaatggaaagtatataaagacaccccctggagtagcagcaccttctgaccctttgctttgcaaatttgctgacggtgggccaaagaaacgacagagccaaggaagatacgtgcaaaatggacgggcctggccaaggaacggagacatgggcggtatggccttgacctatgaccccactgctgcccttcagaatgggttctacgcagctccttacagtatcgcccacagcaggatgcttgctcaatctgcgctagccccgtatcttccatctcctgtgtcttcctatcagggctcagttctgacaccagggatggaccaccccctctctctccagcctgcctccatgatgggacctcttacccagcaactgggtcacctgtcactcaacagtctgggcacgttcatgccggcagctgctgctatgcatggggcttacatctcccagtacccagctgtgccttcttccagtgtttctgctgaggagagcaatggccagcagaatcaactggcagtggagcccccctcagaccacggggtctatcctttccagttcagcaaataatgaggtccagacctggggagagaagcctatgcagtcctccttgggctccttcctgtggctgatggaacctgaggaatcacgttggtttttttttttgaatgtgctacattcaagatcaaaaagacttttttttcttttgcaaaagaagtttcttgctttgtatttaattgcagcgaacctttctcctaccccaaagacaccagttgaggtgcttctcatcttcgagaggtttgggtatgttgggcttttaaaatggtttaagaacaatcgcagtgctgtgaagtcagtgaaggggcgctgcttgccaggttcagttagggactattttcaatgtgtgttttagatatgcaggcttaaaacttttgttttgcaaagctctcaacacacactttgcacacacccacccacctccctcccacgcactgtttaaggcagggtctcacagtgcagtcctggctggctgacaatgtagaccaggctggctttgaactcagcgatccttcccactctgtctgagtgcaccgccatgcctagctagttgtttttttttttttggttttttttttttcaagacagggtttctctgtgtagccctggctgtcctggcgctcactttgtagaccaagctagcctcgaacttagaaatccacctgcctctgcctcccaagtgctgggattaaaggcgtgcgccaccaccgcccggctagttgttttttaaaacttctccacaatggtctttttttcttttccatttagcttagcctgcctactttgcctttttacaatttttaattttatgaatttgatttaaatttcatgtggaattgggggaagggagagcaacgcacaggtagagaagtgtggcagtagaggttgctttccctctgccctcctggcctaggaggggttagactttgacttcaggaagcagacatgtgacaaccatgcagcctttggaaaccaccttcaaccaactctggtggcaagtgccactgagaagtggcatccagcttcagcatcctggatacctgctctgcctcctggagggtcttgggtcttcatcctgccccaggtctcacagcccctgcccctgctgagcaagttctgccttccactttaccaggaggttgttttgtccccgagaggctgctgtcttgtccatcatcatccttgattaccaagcctggggagtatcatgtgtgctggtcctgaacacctgacagaacctggccccactcctccaccccttattccctggcagttatttggtgtagactaaaccccagtccagccttggacatggagcctgttagttcatgtacttggccagcagtgacatctgtgactttgcctcctggaggatcttttctgcctgggttctcacagcctctcatcccagctgcacatggctgtactcaagtggtacttggctgaatcacttaattcagcaggagccatcttatttagcagggctcacccttggttgtatgtacatgccaagtgcacacagtttgaagggatgaaagcaagaactgttgtgtatactgtgcatgcttgagaatggactgagctttctctatgcagcatacccagcccagccctggtgtttggaccccttccccagggaaccagaccaccagaaataattttccttcttgtggaaggacgacggggtgctaggatagaaaaaggcaagactcacagctccctggccactcaaaggtcaggagggacttgtaaacatgcctgccgttaactattcccttctgcaagactttcagcacaaaatgtgacttgttacatcacatcccttcacgtcataagtacacctccagtagacaaagcaatggagatggggaagtgtgtccagaggtcagtgtgaaagaggaagggcagggcatggtgatggtgagaaactggctcagcagctgtgcacactacagaattgggaatcctggcctgactgtgctgctgtgcgttctagactgaggaaggggctgaggacaatggacagcataaagtacaaaatgaccagttttctcattggtgcttccaacatcaggaaggtcatacccagttatcgacctctagccctctagcactcagtgacagactcagagctctgtcctgtggaaaccctgctgacagtcttgctgccactgctgctccttcactgcctattaaaaattgttcctttttctgtagttctaaagcaatttgaataactgacagttttaaaatttgaaattacctttttaggtttttcttttgagtatactggttagggttctagtgtttctggttgaacaggtgtgagcatgggaaatgagggcaacctgtaattttgtttttatagtggttaatggcactcactgtgtaatttctgcttagtgatttccatccactcttttcctcattagctcattactcagaaaggtagcgactgaagacaggaagtagtatgcaagccatgagggatgagttgtaagcctcctctccatcatcctgcccaaggctcctaacagtctcctgagtcctgtttgcatggaggccagatagatggctctgcactctatatctcacctgtactcattttagtacattgtggttttgcttccaatcaatcagagtggactagagctcacacctgacctcgtgtgactcttcactaggctccaggcctatcccatctcattgggtcagactgtagatggactggacttttggagacaggtcctgctattacttaggaatatgtgggaacaatgatagggaccaagcttgtgaagcaaaacggctttggaaagggcaagtgctcaataataaaaaatggggtggaagtgaagcgttatttgctgagggtttcggaaggactagtttgtttttgtccctggcccttccggtcaagtgggcacctcccattttgtcgccaagagcaatacagttgagtaggtggtagacccaaactcacccagccatttctagacctgaattcagaggataaggtgagtctagaggtatatacaaccaatgcttgttagaccaattcttaccaattcggagcaagccggtggctctacttctgggtaacctgcctcttaaaagtgcctttgatcccagtagtagattcagggtctacaggagccttccctcagcagctaaaaccaatttgtctcctctactctttgctgcacctcccggaggtggtctccatgtggcagtgatgccctcatcacccttgtgaccaccgctctgaatgttcaaaataagcatttcctgtccaagcaaatccctaaactccctcgtcctcattactcaactacctcagtctgacaactcaaggcacacaagcacctacttgcctcccaccatcctttactgcccttgtctttgtggggttggaacaaatgcaaactcctcagttccacaacccaaaactgctctttctggatcgtcttctccagtgacgttggctccctacaagagcgaactctccatatgggtcagtccctgtaggacaagccagggactatgctgtgcagtcaaatgccaggtttggagcatagcttaagaccgcagagagtaaggacttgagtggtggtggtgtgcagtttgagagagctggaatggacgtctctgctcctgccctctgggcgggtcgggtgatgacttctagatgcactccttaccctggagggaagttaatttatacttaagatgcattttgtacatttcccctttacccagaaacctgtagtttcatactcccatgtctatgccaacactacctatcgctcactctccgtggctgacttctggttccatttccttcctgtgacttggaagagctttacttttgctcacgtgaacctttcttttttaaataaaacacaaaagcctcc

SEQ ID NO: 8 - RNA, 21 nt, Artificial Sequence
  source 1..21: mol_type = other RNA
tttgcacaaattttccttggt

SEQ ID NO: 9 - RNA, 21 nt, Artificial Sequence
  source 1..21: mol_type = other RNA
taaggagctgcgtagaaccca

SEQ ID NO: 10 - RNA, 21 nt, Artificial Sequence
  source 1..21: mol_type = other RNA
taaggagctgcgtagaaccca

SEQ ID NO: 11 - RNA, 21 nt, Artificial Sequence
  source 1..21: mol_type = other RNA
agatgtataagtttgtagggt

SEQ ID NO: 12 - DNA, 20 bp, Artificial Sequence
  source 1..20: mol_type = other DNA
catctctccctcagcagcac

SEQ ID NO: 13 - DNA, 20 bp, Artificial Sequence
  source 1..20: mol_type = other DNA
gctgctctcctcgactgaaa

SEQ ID NO: 14 - DNA, 20 bp, Artificial Sequence
  source 1..20: mol_type = other DNA
ctccaggagcccagctatga

SEQ ID NO: 15 - DNA, 20 bp, Artificial Sequence
  source 1..20: mol_type = other DNA
gaggtgagtggctgtctgtg

SEQ ID NO: 16 - DNA, 20 bp, Artificial Sequence
  source 1..20: mol_type = other DNA
gaaatgtccgttcggttggc

SEQ ID NO: 17 - DNA, 20 bp, Artificial Sequence
  source 1..20: mol_type = other DNA
tccgataaataacgcgccca

SEQ ID NO: 18 - DNA, 20 bp, Artificial Sequence
  source 1..20: mol_type = other DNA
cgaggcacaaggcacaacag

SEQ ID NO: 19 - DNA, 20 bp, Artificial Sequence
  source 1..20: mol_type = other DNA
agaggtccaggtcctggaag

SEQ ID NO: 20 - DNA, 20 bp, Artificial Sequence
  source 1..20: mol_type = other DNA
gttccacccgcagtacagaa

SEQ ID NO: 21 - DNA, 20 bp, Artificial Sequence
  source 1..20: mol_type = other DNA
agggcttcagcataaagcgt

SEQ ID NO: 22 - DNA, 20 bp, Artificial Sequence
  source 1..20: mol_type = other DNA
accggaaggaaccatctcac

SEQ ID NO: 23 - DNA, 21 bp, Artificial Sequence
  source 1..21: mol_type = other DNA
ggcaaaactgcaccttcacac

SEQ ID NO: 24 - DNA, 20 bp, Artificial Sequence
  source 1..20: mol_type = other DNA
gggccagctgacactagaaa

SEQ ID NO: 25 - DNA, 20 bp, Artificial Sequence
  source 1..20: mol_type = other DNA
gtcatcatagggcagctcgt

SEQ ID NO: 26 - DNA, 20 bp, Artificial Sequence
  source 1..20: mol_type = other DNA
gtctgacgggatcgtggttt

SEQ ID NO: 27 - DNA, 20 bp, Artificial Sequence
  source 1..20: mol_type = other DNA
cagggggcataaacttgtca

SEQ ID NO: 28 - DNA, 21 bp, Artificial Sequence
  source 1..21: mol_type = other DNA
tgctgctatcagtgacttcca

SEQ ID NO: 29 - DNA, 22 bp, Artificial Sequence
  source 1..22: mol_type = other DNA
tgctgagccacatatagcttct

SEQ ID NO: 30 - DNA, 20 bp, Artificial Sequence
  source 1..20: mol_type = other DNA
aggcataacgcactaggttt

SEQ ID NO: 31 - DNA, 20 bp, Artificial Sequence
  source 1..20: mol_type = other DNA
agctggagtcacagaaggag

SEQ ID NO: 32 - DNA, 25 bp, Artificial Sequence
  source 1..25: mol_type = other DNA
caaccaacaagtgatattctccatg

SEQ ID NO: 33 - DNA, 21 bp, Artificial Sequence
  source 1..21: mol_type = other DNA
gatccacactctccagctgca

SEQ ID NO: 34 - DNA, 20 bp, Artificial Sequence
  source 1..20: mol_type = other DNA
atggcctccctctcatcagt

SEQ ID NO: 35 - DNA, 20 bp, Artificial Sequence
  source 1..20: mol_type = other DNA
cttggtggtttgctacgacg

SEQ ID NO: 36 - DNA, 1240 bp, Artificial Sequence
  source 1..1240: mol_type = other DNA
cctactttcagcctggaatcattctgaatgctagctagatatctggagacaggtggacagaaaaccaggaactagtctgaaaaagaaactaaccaaagggaagaagtctgtttaagtttgacccagcctagaagacttgagcattggaggggttattcagagtgagacgtaccaccttcagattcaaatcctgtcatccagtagaagggagcttcaaacacaagctagctaagatacaatgaggtccttcttcgatatctttatcttccatataccatgaatcaaagaaacttcaacaacatgaggactgcaacagaccttcaagcctccttgcatgacctggaaatgttttggggtgtcctggcagcagtgggatcagcactaacagataagggcaactctcacagagactaaaggtcttaactaagaagatagccaagagaccactggggagaatgcagagaataggcttggacttggaagccaagattgcttgacaacagacagaagatatttctgtacttcacccactttacccacctggcaactcctggaaacaactgcacaaaatttggaggtgaacaaaccattagaaacaactggtcctgacaagacacaggaaaaacaagcaatatgcaacattactgtctgttgtccaggttgggtgctgggggtgggagagggagtgtgtgtctttgtatgatctgaaaaaactcaggtcagaacatctgtagatccttacagacatacaaaagaatcctagcctcttattcatgtgtgtgtgtgtgtgtgtgtgtgtgtgtgtgtgtgtgtgtgtgtgtatgtgtgtgtcgtctgtcatgcgcgcgtgcctgcgtttaaataacatcagctttagcttctctttctccttataaaacattgtgaatttcagttttctttcccatcaagacatgctcaagtgctgagtcacttttaaagaaaaaaaagaagagtgctcatgcttcttagggctagcctcaaggatgacttaagcacactttccccttcctagttgtgattctttcgatgctaaacgacgtcacattgtgcaatcttaataaggtttccaatcagccccacccactctggccccacccccaccctccaacaaagatttttatcaaatgtgggattttcccatgagtctcaaaattagagagttgactcctaataaatatgagactggggatgtctgtagctcattctgctctggagccca

SEQ ID NO: 37 - DNA, 171 bp, Artificial Sequence
  source 1..171: mol_type = other DNA
ctaaaagtatgagcgttaggacactattttaattatttttaatttattaatatttaaatatgtgaagctgagttaatttatgtaagtcatatttatatttttaagaagtaccacttgaaacattttatgtattagttttgaaataataatggaaagtggctatgcagtttg

SEQ ID NO: 38 - DNA, 72 bp, Artificial Sequence
  source 1..72: mol_type = other DNA
tattttaattatttttaatttattaatatttaaatatgtgaagctgagttaatttatgtaagtcatatttat

SEQ ID NO: 39 - DNA, 39 bp, Artificial Sequence
  source 1..39: mol_type = other DNA
tattttaattatttttaatttattaatatttaaatatgt

SEQ ID NO: 40 - DNA, 101 bp, Artificial Sequence
  source 1..101: mol_type = other DNA
agttaatttatgtaagtcatatttatatttttaagaagtaccacttgaaacattttatgtattagttttgaaataataatggaaagtggctatgcagtttg

SEQ ID NO: 41 - DNA, 71 bp, Artificial Sequence
  source 1..71: mol_type = other DNA
tattttaattatttttaagggattaatagggaaatatgtgaagctgagttaagggatgtaagtcataggga

SEQ ID NO: 42 - DNA, 357 bp, Artificial Sequence
  source 1..357: mol_type = other DNA
ggatccacaagtccttgttccactgtgccttggtttctcctttatttctaagtggaaaaagtattagccaccatcttacctcacagtgatgttgtgaggacatgtggaagcactttaagttttttcatcataacataaattattttcaagtgtaacttattaacctatttattatttatgtatttatttaagcatcaaatatttgtgcaagaatttggaaaaatagaagatgaatcattgattgaatagttataaagatgttatagtaaatttattttattttagatattaaatgatgttttattagataaatttcaatcagggtttttagattaaacaaacaaacaattgggtacc

SEQ ID NO: 43 - DNA, 357 bp, Artificial Sequence
  source 1..357: mol_type = other DNA
ggatccacaagtccttgttccactgtgccttggtttctcctttatttctaagtggaaaaagtattagccaccatcttacctcacagtgatgttgtgaggacatgtggaagcactttaagttttttcatcataacataaattattttcaagtgtaacttattaacctagggattagggatgtagggagggaagcatcaaatatttgtgcaagaatttggaaaaatagaagatgaatcattgattgaatagttataaagatgttatagtaaatttattttattttagatattaaatgatgttttattagataaatttcaatcagggtttttagattaaacaaacaaacaattgggtacc

SEQ ID NO: 44 - DNA, 584 bp, Artificial Sequence
  source 1..584: mol_type = other DNA
agagagctgtacccagagagtcctgtgctgaatgtggactcaatccctagggctggcagaaagggaacagaaaggtttttgagtacggctatagcctggactttcctgttgtctacaccaatgcccaactgcctgccttagggtagtgctaagaggatctcctgtccatcagccaggacagtcagctctctcctttcagggccaatccccagcccttttgttgagccaggcctctctcacctctcctactcacttaaagcccgcctgacagaaaccacggccacatttggttctaagaaaccctctgtcattcgctcccacattctgatgagcaaccgcttccctatttatttatttatttgtttgtttgttttattcattggtctaatttattcaaagggggcaagaagtagcagtgtctgtaaaagagcctagtttttaatagctatggaatcaattcaatttggactggtgtgctctctttaaatcaagtcctttaattaagactgaaaatatataagctcagattatttaaatgggaatatttataaatgagcaaatatcatactgttcaatggttctga

SEQ ID NO: 45 - DNA, 584 bp, Artificial Sequence; identical to SEQ ID NO: 44
  source 1..584: mol_type = other DNA

SEQ ID NO: 46 - protein, 304 aa, Artificial Sequence
MDYKDHDGDYKDHDIDYKDDDDKKLLEEQDPTNLYISNLPLSMDEQELEGMLKPFGQVISTRILRDTSGTSRGVGFARMESTEKCEAIITHFNGKYIKTPPGVPAPSDPLLCKFADGGPKKRQNQGKFVQNGRAWPRNADMGVMALTYDPTTALQNGFYPAPYNITPNRMLAQSALSPYLSSPVSSYQRVTQTSPLQVPNPSWMHHHSYLMQPSGSVLTPGMDHPISLQPASMMGPLTQQLGHLSLSSTGTYMPTAAAMQGAYISQYTPVPSSSVSVEESSGQQNQVAVDAPSEHGVYSFQFNK

SEQ ID NO: 47 - protein, 321 aa, Artificial Sequence
MDYKDHDGDYKDHDIDYKDDDDKKLAPPSPSNSTPNSSSGSNGNDQLSKTNLYIRGLQPGTTDQDLVKLCQPYGKIVSTKAILDKTTNKCKGYGFVDFDSPSAAQKAVTALKASGVQAQMAKQQEQDPCKFADGGPKKRQNQGKFVQNGRAWPRNADMGVMALTYDPTTALQNGFYPAPYNITPNRMLAQSALSPYLSSPVSSYQRVTQTSPLQVPNPSWMHHHSYLMQPSGSVLTPGMDHPISLQPASMMGPLTQQLGHLSLSSTGTYMPTAAAMQGAYISQYTPVPSSSVSVEESSGQQNQVAVDAPSEHGVYSFQFNK

SEQ ID NO: 48 - protein, 216 aa, Artificial Sequence
MDYKDHDGDYKDHDIDYKDDDDKKLLEDGGPKKRQNQGKFVQNGRAWPRNADMGVMALTYDPTTALQNGFYPAPYNITPNRMLAQSALSPYLSSPVSSYQRVTQTSPLQVPNPSWMHHHSYLMQPSGSVLTPGMDHPISLQPASMMGPLTQQLGHLSLSSTGTYMPTAAAMQGAYISQYTPVPSSSVSVEESSGQQNQVAVDAPSEHGVYSFQFNK